European Patent Application EP 4 534 646 A1, published April 9, 2025. Title: CEPAS DE LEVADURA CON PROPIEDADES VINÍCOLAS OPTIMIZADAS Y SU MÉTODO DE OBTENCIÓN. Applicant: UNIVERSITAT POLITECNICA DE VALENCIA. Application ES. The sequence listing filed with the application follows.

SEQUENCE LISTING (8 sequences)

SEQ ID NO: 1 - DNA, 1767 bp, Saccharomyces cerevisiae
  source 1..1767: mol_type = genomic DNA
atgtcaacacttagcgatagtgataccgagactgaggtcgtgtcgagaaacttgtgtggaatcgtcgacataggttctaatggtattcgttttagtatatcttccaaggctgcacatcatgcaagaattatgccttgtgtttttaaagatagggttggtctttctctatacgaagttcaatataatacacatacgaacgcaaaatgccctattcccagagatattataaaagaggtttgttctgccatgaagagattcaaattaatttgcgatgattttggtgtacctgaaactagtgtcagagtaattgcaacagaagccacgcgagatgctattaacgcggatgaatttgttaatgctgtttacggtagcactggctggaaagtagaaatattaggccaggaagatgaaactagggtcggcatatatggtgttgtttcctcatttaatacagtaagaggtctatatctagatgtggcaggtggtagtactcagttatcatgggtaataagctcgcacggagaagtcaagcaatccagcaaacctgtatctttgccatatggagctggaactcttttgagaagaatgagaacagatgataatagggcacttttttatgagattaaagaagcgtacaaagatgcgattgaaaaaattggtatacctcaagaaatgattgatgacgccaagaaagaaggtggatttgacctttggacccgtgggggtggtttaagaggtatgggacatctgcttctttaccagtcggaaggttatcccatccaaacaataattaacggatatgcttgcacttatgaagaattctcgtctatgtcagattatctattcctaaaacaaaaaataccaggttcttcaaaagagcataaaatatttaaggtttctgatagaagggctttacaacttcctgccgttggtttgttcatgagtgctgtttttgaagcgattccccagatcaaagctgtacattttagtgagggtggtgttcgagagggttcactttattctcttcttccaaaagaaattcgtgcacaagatccattgctaattgcgtcccgtccttatgctccattacttactgaaaaatatctatatctattgagaacatcaatcccacaagaagatataccagaaatagtaaacgaaaggattgctcctgctttatgtaacttagcatttgttcatgcctcttatccaaaggagttacaaccaacagctgcattacatgttgctacaagagggataatagccggctgtcatggattatctcacagagctagagcgctgataggaattgctctatgtagtagatggggcggcaacattccggaatctgaagaaaaatactcccaagaattagaacaagtagttctacgcgaaggtgataaagctgaagcattgagaattgtatggtggacgaagtatattggtacgattatgtatgtgatttgcggtgttcatccaggtggtaatatcagagataacgtatttgatttccatgtttctaagcgtagtgaggtggagaccagtttaaaagaattaatcattgatgatgcaaacactacaaaggtaaaagaagaatccacgcgtaaaaatcgcgggtatgaagtggttgtgagaattagtaaggacgatcttaaaacaagtgcttccgttcgttccagaattatcacgctacaaaagaaagtacgcaagctatctagaggaagtgtagagagggttaaaattggcgtgcaattttatgaagaataa

SEQ ID NO: 2 - DNA, 1767 bp, Saccharomyces cerevisiae
  source 1..1767: mol_type = genomic DNA
atgtcaacacttagcgatagtgataccgagactgaggtcgtgtcgagaaacttgtgtggaatcgtcgacataggttctaatggtattcgttttagtatatcttccaaggctgcacatcatgcaagaattatgccttgtgtttttaaagatagggttggtctttctctatacgaagttcaatataatacacatacgaacgcaaaatgccctattcccagagatattataaaagaggtttgttctgccatgaagagattcaaattaatttgcgatgattttggtgtacctgaaactagtgtcagagtaattgcaacagaagccacgcgagatgctattaacgcggatgaatttgttaatgctgtttacggtagcactggctggaaagtagaaatattaggccaggaagatgaaactagggtcggcatatatggtgttgtttcctcatttaatacagtaagaggtctatatctagatgtggcaggtggtagtactcagttatcatgggtaataagctcgcacggagaagtcaagcaatccagcaaacctgtatctttgccatatggagctggaactcttttgagaagaatgagaacagatgataatagggcacttttttatgagattaaagaagcgtacaaagatgcgattgaaaaaattggtatacctcaagaaatgattgatgacgccaagaaagaaggtggatttgacctttggacccgtgggggtggtttaagaggtatggaacatctgcttctttaccagtcggaaggttatcccatccaaacaataattaacggatatgcttgcacttatgaagaattctcgtctatgtcagattatctattcctaaaacaaaaaataccaggttcttcaaaagagcataaaatatttaaggtttctgatagaagggctttacaacttcctgccgttggtttgttcatgagtgctgtttttgaagcgattccccagatcaaagctgtacattttagtgagggtggtgttcgagagggttcactttattctcttcttccaaaagaaattcgtgcacaagatccattgctaattgcgtcccgtccttatgctccattacttactgaaaaatatctatatctattgagaacatcaatcccacaagaagatataccagaaatagtaaacgaaaggattgctcctgctttatgtaacttagcatttgttcatgcctcttatccaaaggagttacaaccaacagctgcattacatgttgctacaagagggataatagccggctgtcatggattatctcacagagctagagcgctgataggaattgctctatgtagtagatggggcggcaacattccggaatctgaagaaaaatactcccaagaattagaacaagtagttctacgcgaaggtgataaagctgaagcattgagaattgtatggtggacgaagtatattggtacgattatgtatgtgatttgcggtgttcatccaggtggtaatatcagagataacgtatttgatttccatgtttctaagcgtagtgaggtggagaccagtttaaaagaattaatcattgatgatgcaaacactacaaaggtaaaagaagaatccacgcgtaaaaatcgcgggtatgaagtggttgtgagaattagtaaggacgatcttaaaacaagtgcttccgttcgttccagaattatcacgctacaaaagaaagtacgcaagctatctagaggaagtgtagagagggttaaaattggcgtgcaattttatgaagaataa

SEQ ID NO: 3 - DNA, 1767 bp, Saccharomyces cerevisiae
  source 1..1767: mol_type = genomic DNA
atgtcaacacttagcgatagtgataccgagactgaggtcgtgtcgagaaacttgtgtggaatcgtcgacataggttctaatggtatttgttttagtatatcttccaaggctgcacatcatgcaagaattatgccttgtgtttttaaagatagggttggtctttctctatacgaagttcaatataatacacatacgaacgcaaaatgccctattcccagagatattataaaagaggtttgttctgccatgaagagattcaaattaatttgcgatgattttggtgtacctgaaactagtgtcagagtaattgcaacagaagccacgcgagatgctattaacgcggatgaatttgttaatgctgtttacggtagcactggctggaaagtagaaatattaggccaggaagatgaaactagggtcggcatatatggtgttgtttcctcatttaatacagtaagaggtctatatctagatgtggcaggtggtagtactcagttatcatgggtaataagctcgcacggagaagtcaagcaatccagcaaacctgtatctttgccatatggagctggaactcttttgagaagaatgagaacagatgataatagggcacttttttatgagattaaagaagcgtacaaagatgcgattgaaaaaattggtatacctcaagaaatgattgatgacgccaagaaagaaggtggatttgacctttggacccgtgggggtggtttaagaggtatggaacatctgcttctttaccagtcggaaggttatcccatccaaacaataattaacggatatgcttgcacttatgaagaattctcgtctatgtcagattatctattcctaaaacaaaaaataccaggttcttcaaaagagcataaaatatttaaggtttctgatagaagggctttacaacttcctgccgttggtttgttcatgagtgctgtttttgaagcgattccccagatcaaagctgtacattttagtgagggtggtgttcgagagggttcactttattctcttcttccaaaagaaattcgtgcacaagatccattgctaattgcgtcccgtccttatgctccattacttactgaaaaatatctatatctattgagaacatcaatcccacaagaagatataccagaaatagtaaacgaaaggattgctcctgctttatgtaacttagcatttgttcatgcctcttatccaaaggagttacaaccaacagctgcattacatgttgctacaagagggataatagccggctgtcatggattatctcacagagctagagcgctgataggaattgctctatgtagtagatggggcggcaacattccggaatctgaagaaaaatactcccaagaattagaacaagtagttctacgcgaaggtgataaagctgaagcattgagaattgtatggtggacgaagtatattggtacgattatgtatgtgatttgcggtgttcatccaggtggtaatatcagagataacgtatttgatttccatgtttctaagcgtagtgaggtggagaccagtttaaaagaattaatcattgatgatgcaaacactacaaaggtaaaagaagaatccacgcgtaaaaatcgcgggtatgaagtggttgtgagaattagtaaggacgatcttaaaacaagtgcttccgttcgttccagaattatcacgctacaaaagaaagtacgcaagctatctagaggaagtgtagagagggttaaaattggcgtgcaattttatgaagaataa

SEQ ID NO: 4 - DNA, 1767 bp, Saccharomyces cerevisiae
  source 1..1767: mol_type = genomic DNA
atgtcaacacttagcgatagtgataccgagactgaggtcgtgtcgagaaacttgtgtggaatcgtcgacataggttctaatggtattcgttttagtatatcttccaaggctgcacatcatgcaagaattatgccttgtgtctttaaagatagggttggtctttctctatacgaagttcaatataatacacatacgaacgcaaaatgccctattcccagagatattataaaagaggtttgttctgccatgaagagattcaaattaatttgcgatgattttggtgtacctgaaactagtgtcagagtaattgcaacagaagccacgcgagatgctattaacgcggatgaatttgttaatgctgtttacggtagcactggctggaaagtagaaatattaggccaggaagatgaaactagggtcggcatatatggtgttgtttcctcatttaatacagtaagaggtctatatctagatgtggcaggcggtagtactcagttatcatgggtaataagctcgcacggagaagtcaagcaatccagcaaacctgtatctttgccatatggagctggaactcttttgagaagaatgagaacagatgataatagggcacttttttatgagattaaagaagcgtacaaagatgcgattgaaaaaattggtatacctcaagaaatgattgatgatgccaagaaagaaggtggatttgacctttggacccgtgggggtggtttaagaggtatgggacatctgcttctttaccagtcggaaggttatcccatccaaacaataattaacggatatgcttgcacttatgaagaattctcgtctatgtcagattatctattcctaaaacaaaaaataccaggttcttcaaaagagcataaaatatttaaggtttctgatagaagggctttacaacttcctgccgttggtttgttcatgagtgctgtttttgaagcgattccccagatcaaagctgtacattttagtgagggtggtgttcgagagggttcactttattctcttcttccaaaagaaattcgtgcacaagatccattgctaattgcgtcccgtccttatgctccattacttactgaaaaatatctatatctattgagaaaatcaatcccacaagaagatataccagaaatagtaaacgaaaggattgctcctgctttatgtaacttagcatttgttcatgcctcttatccaaaggagttacaaccaacagctgcattacatgttgctacaagagggataatagccggctgtcatggattatctcacagagctagagcgctgataggaattgctctatgtagtagatggggcggcaacattccggaatctgaagaaaaatactcccaagaattagaacaagtagttctacgcgaaggtgataaagctgaagcattgagaattgtatggtggacgaagtatattggtacgattatgtatgtgatttgcggtgttcatccaggtggtaatatcagagataacgtatttgatttccatgtttctaagcgtagtgaggtggagaccagtttaaaagaattaatcattgatgatgcaaacactacaaaggtaaaagaagaatccacgcgtaaaaatcgcgggtatgaagtggttgtgagaattagtaaggacgatcttaaaacaagtgcttccgttcgttccaaaattatcacgctacaaaagaaagtacgcaagctatctagaggaagtgtagagagggttaaaattggcgtgcaattttatgaagaataa

SEQ ID NO: 5 - DNA, 1323 bp, Saccharomyces cerevisiae
  source 1..1323: mol_type = genomic DNA
atgtctgaaaataacgaattccagagtgtcaccgaatcgacgactgctccaaccactagtaacccatatggcccaaatcctgcggattatctatccaatgttaagaatttccagttgattgattcaacactaagagagggtgaacaatttgccaacgcattcttcgatactgaaaaaaagattgaaattgctagagccttggatgatttcggtgtggactacatcgagttaacctctcccgtagcatccgaacaatcaagaaaggactgtgaagctatatgtaaactaggtttaaaggccaagatccttacacacattcgttgtcacatggacgatgccagagtcgccgtagagactggtgtcgacggtgtcgatgttgttatcggcacctccaaatttttaagacaatattcccacggtaaggatatgaactacatcgccaagagtgctgttgaagtcattgaatttgtcaaatccaaaggtattgaaatcagattttcctctgaagattccttcagaagtgatctcgttgatcttttgaacatttataaaaccgttgacaagatcggtgtaaatagagtcggtattgccgacacagttggatgtgccaacccaagacaagtatatgaactgatcagaactttgaagagtgttgtctcatgtgacatcgaatgccatttccacaatgataccggttgtgccattgcaaacgcctacactgctttggaaggtggtgccagattgattgacgtcagtgtactgggtattggtgaaagaaacggtatcactcctctaggtgggctcatggcaagaatgattgttgccgcaccagactatgtcagatctaaatacaagctgcacaagatcagagacatcgaaaacctggtcgctgatgctgtggaagttaacattccattcaacaaccctatcaccgggttctgtgcattcacacataaagcaggtatccatgccaaggccattttggctaacccatctacctacgaaatcttggaccctcacgatttcggtatgaagagatatatccacttcgccaacagactaactggttggaatgcaatcaaatcaagagtcgaccaattgaacttgaatttgacggatgatcaaatcaaggaagttactgctaagattaagaagctgggtgatgtcagaccgctaaatattgatgatgtagactccattatcaaggacttccatgcagaattgagcaccccacttttaaaaccagtaaataagggtacagatgacgacaatatcgatatttccaatgggcatgtttctaaaaaggcaaaggtcaccaaatag

SEQ ID NO: 6 - DNA, 1323 bp, Saccharomyces cerevisiae
  source 1..1323: mol_type = genomic DNA
atgtctgaaaataacgaattccagagtgtcaccgaatcgacgactgctccaaccactagtaacccatatggcccaaatcctgcggattatctatccaatgttaagaatttccagttgattgattcaacactaagagagggtgaacaatttgccaacgcattcttcgatactgaaaaaaagattgaaattgctagagccttggatgatttcggtgtggactacatcgagttaacctctcccgtagcatccgaacaatcaagaaaggactgtgaagctatatgtaaactaggtttaaaggccaagatccttacacacattcgttgtcacatggacgatgccagagtcgccgtagagactggtgtcgacggtgtcgatgttgttatcggcacctccaaatttttaagacaatattcccacggtaaggatatgaactacatcgccaagagtgctgttgaagtcattgaatttgtcaaatccaaaggtattgaaatcagattttcctctgaagattccttcagaagtgatctcgttgatcttttgaacatttataaaaccgttgacaagatcggtgtaaatagagtcggtattgccgacacagttggatgtgccaacccaagacaagtatatgaactgatcagaactttgaagagtgttgtctcatgtgacatcgaatgccatttccacaatgataccggttgtgccattgcaaacgcctacactgctttggaaggtggtgccagattgattgacgtcagtgtactgggtattggtgaaagaaacggtatcactcctctaggtgggctcatggcaagaatgattgttgccgcaccagactatgtcagatctaaatacaagctgcacaagatcagagacatcgaaaacctggtcgctgatgctgtggaagttaacattccattcaacaaccctatcaccgggttctgtgcattcacacataaagcaggtatccatgccaaggccattttggctaacccatctacctacgaaatcttggaccctcacgatttcggtatgaagagatatatccacttcgccaacagactaactggttggaatgcaatcaaatcaagagtcgaccaattgaacttgaatttgacggatgatcaaatcaaggaagttactgctaagattaagaagctgggtgatgtcggaccgctaaatattgatgatgtagactccattatcaaggacttccatgcagaattgagcaccccacttttaaaaccagtaaataagggtacagatgacgacaatatcgatatttccaatgggcatgtttctaaaaaggcaaaggtcaccaaatag

SEQ ID NO: 7 - DNA, 1287 bp, Saccharomyces cerevisiae
  source 1..1287: mol_type = genomic DNA
atgactgctgctaaaccaaatccatatgctgccaaaccgggcgactatctttctaatgtaaataatttccagttaatcgattcgacgctgagagaaggtgaacaatttgccaacgcattcttcgatactgaaaaaaagatcgaaattgctagagccttggacgatttcggtgtggactacatcgagttaacctcaccagtagcatctgaacaatcaagaaaggactgtgaagctatatgtaaactaggtttaaaggccaagatccttacacacattcgttgtcatatggatgacgccaaagtcgccgtagagactggtgtcgacggtgtcgatgtcgttatcggcacctccaaatttttaagacaatattcccacggtaaggatatgaactacatcgccaagagtgctgttgaagtcattgaatttgtcaaatccaaaggtattgaaatcagattttcctctgaagattccttcagaagtgatctcgttgatcttttgaacatttataaaaccgttgacaagatcggtgtaaatagagtcggtattgccgacacagttggatgtgccaacccaagacaagtatatgaactgatcagaactttgaagagtgttgtttcatgtgacatcgaatgccatttccacaacgatactggttgtgccattgcaaacgcctacactgctttggaaggtggtgccagattgattgacgtcagtgtactgggtattggtgaaagaaacggtatcactcctctaggtgggctcatggcaagaatgattgttgccgcaccagactatgtcaagtccaaatacaagttgcacaagatcagagacattgaaaacctggtcgctgatgctgtggaagttaacattccattcaacaaccctatcaccgggttctgtgcattcacacataaagcaggtatccatgccaaggccattttggctaacccatctacctacgaaatcttggaccctcacgatttcggtatgaagaggtatatccacttcgccaacagactaactggctggaacgccatcaaagccagagtcgaccagttgaacttgaacttgacggatgaccaaatcaaggaagttactgctaagattaagaagctgggtgatgtcagatcgctgaatatcgatgatgttgactctatcatcaagaacttccacgcagaggtcagcactcctcaagtactatctgcaaaaaagaacaagaagaatgacagcgatgtaccggaactggccaccatccccgccgccaagcggactaagccatccgcctaa

SEQ ID NO: 8 - DNA, 1287 bp, Saccharomyces cerevisiae
  source 1..1287: mol_type = genomic DNA
atgactgctgctaaaccaaatccatatgctgccaaaccgggcgactatctttctaatgtaaataatttccagttaatcgattcgacgctgagagaaggtgaacaatttgccaacgcattcttcgatactgaaaaaaagatcgaaattgctagagccttggacgatttcggtgtggactacatcgagttaacctcaccagtagcatctgaacaatcaagaaaggactgtgaagctatatgtaaactaggtttaaaggccaagatccttacacacattcgttgtcatatggatgacgccaaagtcgccgtagagactggtgtcgacggtgtcgatgtcgttatcggcacctccaaatttttaagacaatattcccacggtaaggatatgaactacatcgccaagagtgctgttgaagtcattgaatttgtcaaatccaaaggtattgaaatcagattttcctctgaagattccttcagaagtgatctcgttgatcttttgaacatttataaaaccgttgacaagatcggtgtaaatagagtcggtattgccgacacagttggatgtgccaacccaagacaagtatatgaactgatcagaactttgaagagtgttgtttcatgtgacatcgaatgccatttccacaacgatactggttgtgccattgcaaacgcctacactgctttggaaggtggtgccagattgattgacgtcagtgtactgggtattggtgaaagaaacggtatcactcctctaggtgggctcatggcaagaatgattgttgccgcaccagactatgtcaagtccaaatacaagttgcacaagatcagagacattgaaaacctggtcgctgatgctgtggaagttaacattccattcaacaaccctatcaccgggttctgtgcattcacacataaagcaggtatccatgccaaggccattttggctaacccatctacctacgaaatcttggaccctcacgatttcggtatgaagaggtatatccacttcgccaacagactaactggctggaacgccatcaaagccagagtcgaccagttgaacttgaacttgacggatgaccaaatcaaggaagttactgctaagattaagaagctgggtgatgtcagatcgctggatatcgatgatgttgactctatcatcaagaacttccacgcagaggtcagcactcctcaagtactatctgcaaaaaagaacaagaagaatgacagcgatgtaccggaactggccaccatccccgccgccaagcggactaagccatccgcctaa